European Patent Application EP 4 585 612 A1, published July 16, 2025. Title: FUSION PROTEINS CONTAINING CITOMEGALOVIRUS US6 PROTEIN. Applicant: FUNDACIÓ DE RECERCA CLINIC BARCELONA-INSTITUT D'INVESTIGACIONS BIOMÈDIQUES AUGUST PI I SUNYER. The sequence listing filed with the application follows.

SEQUENCE LISTING (28 sequences)

SEQ ID NO: 1 - protein, 186 aa, synthetic construct
MKPVLVLAILAVLFLRLADSVPRPLDVVVSEIRSAHFRVEENQCWFHMGMLYFKGRMSGNFTEKHFVNVGIVSQSYMDRLQVSGEQYHHDERGAYFEWNIGGHPVTHTVDMVDITLSTRWGDPKKYAACVPQVRMDYSSQTINWYLQRSMRDDNWGLLFRTLLVYLFSLVVLVLLTVGVSARLRFI

SEQ ID NO: 2 - protein, 183 aa, synthetic construct
MDLLIRLGFLLMCALPTPGERSSRDPKTLLSLSPRQQACVPRTKSHRPVCYNDTGDCTDADDSWKQLGEDFAHQCLQAAKKRPKTHKSRPNDRNLEGRLTCQRVRRLLPCDLDIHPSHRLLTLMNNCVCDGAVWNAFRLIERHGFFAVTLYLCCGITLLVVILALLCSITYESTGRGIRRCGS

SEQ ID NO: 3 - protein, 159 aa, synthetic construct
MRYMILGLLALAAVCSAAKKVEFKEPACNVTFKSEANECTTLIKCTTEHEKLIIRHKDKIGKYAVYAIWQPGDTNDYNVTVFQGENRKTFMYKFPFYEMCDITMYMSKQYKLWPPQKCLENTGTFCSTALLITALALVCTLLYLKYKSRRSFIDEKKMP

SEQ ID NO: 4 - protein, 18 aa, synthetic construct
EGRGSLLTCGDVEENPGP

SEQ ID NO: 5 - protein, 231 aa, synthetic construct
MAQSKHGLTKEMTMKYRMEGCVDGHKFVITGEGIGYPFKGKQAINLCVVEGGPLPFAEDILSAAFMYGNRVFTEYPQDIVDYFKNSCPAGYTWDRSFLFEDGAVCICNADITVSVEENCMYHESKFYGVNFPADGPVMKKMTDNWEPSCEKIIPVPKQGILKGDVSMYLLLKDGGRLRCQFDTVYKAKSVPRKMPDWHFIQHKLTREDRSDAKNQKWHLTEHAIASGSALP

SEQ ID NO: 6 - protein, 107 aa, synthetic construct
DIVMTQSPAIMSASPGEKVTMTCSASSSVSYMNWYQQKSGTSPKRWIYDSSKLASGVPARFSGSGSGTSYSLTISSMETEDAATYYCQQWSRNPPTFGGGTKLQITR

SEQ ID NO: 7 - protein, 120 aa, synthetic construct
QVQLQQSGELARPGASVKMSCKASGYTFTRSTMHWVKQRPGQGLEWIGYINPSSAYTNYNQKFKDKATLTADKSSSTAYMQLSSLTSEDSAVYYCASPQVHYDYNGFPYWGQGTLVTVSS

SEQ ID NO: 8 - protein, 20 aa, synthetic construct
GGGGSGGGGSGGGGSGGGGS

SEQ ID NO: 9 - protein, 21 aa, synthetic construct
MALPVTALLLPLALLLHAARP

SEQ ID NO: 10 - protein, 247 aa, synthetic construct
DIVMTQSPAIMSASPGEKVTMTCSASSSVSYMNWYQQKSGTSPKRWIYDSSKLASGVPARFSGSGSGTSYSLTISSMETEDAATYYCQQWSRNPPTFGGGTKLQITRGGGGSGGGGSGGGGSGGGGSQVQLQQSGELARPGASVKMSCKASGYTFTRSTMHWVKQRPGQGLEWIGYINPSSAYTNYNQKFKDKATLTADKSSSTAYMQLSSLTSEDSAVYYCASPQVHYDYNGFPYWGQGTLVTVSS

SEQ ID NO: 11 - protein, 107 aa, synthetic construct
QIVLTQSPAIMSASPGEKVTMTCSASSSVSYMNWYQQKSGTSPKRWIYDSSKLASGVPARFSGSGSGTSYSLTISSMEAEDAATYYCQQWSRNPPTFGGGTKLEIKR

SEQ ID NO: 12 - protein, 121 aa, synthetic construct
QVQLQQSGAELAKPGASVKMSCKASGYTFTRSTMHWVKQRPGQGLEWIGYINPSSAYTNYNQKFKDKATLTADKSSSTAYMQLSSLTSEDSAVYYCARPQVHYDYNGFPYWGQGTTVTVSS

SEQ ID NO: 13 - protein, 248 aa, synthetic construct
QIVLTQSPAIMSASPGEKVTMTCSASSSVSYMNWYQQKSGTSPKRWIYDSSKLASGVPARFSGSGSGTSYSLTISSMEAEDAATYYCQQWSRNPPTFGGGTKLEIKRGGGGSGGGGSGGGGSGGGGSQVQLQQSGAELAKPGASVKMSCKASGYTFTRSTMHWVKQRPGQGLEWIGYINPSSAYTNYNQKFKDKATLTADKSSSTAYMQLSSLTSEDSAVYYCARPQVHYDYNGFPYWGQGTTVTVSS

SEQ ID NO: 14 - protein, 10 aa, synthetic construct
SASSSVSYMN

SEQ ID NO: 15 - protein, 7 aa, synthetic construct
DSSKLAS

SEQ ID NO: 16 - protein, 9 aa, synthetic construct
QQWSRNPPT

SEQ ID NO: 17 - protein, 10 aa, synthetic construct
GYTFTRSTMH

SEQ ID NO: 18 - protein, 17 aa, synthetic construct
YINPSSAYTNYNQKFKD

SEQ ID NO: 19 - protein, 12 aa, synthetic construct
PQVHYDYNGFPY

SEQ ID NO: 20 - protein, 433 aa, synthetic construct
MALPVTALLLPLALLLHAARPQIVLTQSPAIMSASPGEKVTMTCSASSSVSYMNWYQQKSGTSPKRWIYDSSKLASGVPARFSGSGSGTSYSLTISSMEAEDAATYYCQQWSRNPPTFGGGTKLEIKRGGGGSGGGGSGGGGSGGGGSQVQLQQSGAELAKPGASVKMSCKASGYTFTRSTMHWVKQRPGQGLEWIGYINPSSAYTNYNQKFKDKATLTADKSSSTAYMQLSSLTSEDSAVYYCARPQVHYDYNGFPYWGQGTTVTVSSERSSRDPKTLLSLSPRQQACVPRTKSHRPVCYNDTGDCTDADDSWKQLGEDFAHQCLQAAKKRPKTHKSRPNDRNLEGRLTCQRVRRLLPCDLDIHPSHRLLTLMNNCVCDGAVWNAFRLIERHGFFAVTLYLCCGITLLVVILALLCSITYESTGRGIRRCGS

SEQ ID NO: 21 - protein, 10 aa, synthetic construct
SASSSVSYMN

SEQ ID NO: 22 - protein, 7 aa, synthetic construct
DTSKLAS

SEQ ID NO: 23 - protein, 9 aa, synthetic construct
QQWSSNPFT

SEQ ID NO: 24 - protein, 5 aa, synthetic construct
RYTMH

SEQ ID NO: 25 - protein, 17 aa, synthetic construct
YINPSRGYTNYNQKFKD

SEQ ID NO: 26 - protein, 10 aa, synthetic construct
YYDDHYCLDY

SEQ ID NO: 27 - protein, 247 aa, synthetic construct
EVQLQQSGAELARPGASVKMSCKASGYTFTRYTMHWVKQRPGQGLEWIGYINPSRGYTNYNQKFKDKATLTTDKSSSTAYMQLSSLTSEDSAVYYCARYYDDHYCLDYWGQGTTLTVSSAGGGGSGGGGSGGGGSGGGGSQIVLTQSPAIMSASPGEKVTMTCSASSSVSYMNWYQQKSGTSPKRWIYDTSKLASGVPAHFRGSGSGTSYSLTISGMEAEDAATYYCQQWSSNPFTFGSGTKLEINR

SEQ ID NO: 28 - protein, 432 aa, synthetic construct
MALPVTALLLPLALLLHAARPEVQLQQSGAELARPGASVKMSCKASGYTFTRYTMHWVKQRPGQGLEWIGYINPSRGYTNYNQKFKDKATLTTDKSSSTAYMQLSSLTSEDSAVYYCARYYDDHYCLDYWGQGTTLTVSSAGGGGSGGGGSGGGGSGGGGSQIVLTQSPAIMSASPGEKVTMTCSASSSVSYMNWYQQKSGTSPKRWIYDTSKLASGVPAHFRGSGSGTSYSLTISGMEAEDAATYYCQQWSSNPFTFGSGTKLEINRERSSRDPKTLLSLSPRQQACVPRTKSHRPVCYNDTGDCTDADDSWKQLGEDFAHQCLQAAKKRPKTHKSRPNDRNLEGRLTCQRVRRLLPCDLDIHPSHRLLTLMNNCVCDGAVWNAFRLIERHGFFAVTLYLCCGITLLVVILALLCSITYESTGRGIRRCGS